European Patent Specification EP 3 682 912 B1, published November 26, 2025. Title: USE OF SELF-ASSEMBLING POLYPEPTIDES AS TISSUE ADHESIVES. Applicant: AMsilk GmbH. The sequence listing filed with the application follows.

SEQUENCE LISTING (78 sequences)

SEQ ID NO: 1 - protein, 636 aa, Araneus diadematus
  PEPTIDE (1)..(636): ADF-3
ARAGSGQQGPGQQGPGQQGPGQQGPYGPGASAAAAAAGGYGPGSGQQGPSQQGPGQQGPGGQGPYGPGASAAAAAAGGYGPGSGQQGPGGQGPYGPGSSAAAAAAGGNGPGSGQQGAGQQGPGQQGPGASAAAAAAGGYGPGSGQQGPGQQGPGGQGPYGPGASAAAAAAGGYGPGSGQGPGQQGPGGQGPYGPGASAAAAAAGGYGPGSGQQGPGQQGPGQQGPGGQGPYGPGASAAAAAAGGYGPGYGQQGPGQQGPGGQGPYGPGASAASAASGGYGPGSGQQGPGQQGPGGQGPYGPGASAAAAAAGGYGPGSGQQGPGQQGPGQQGPGQQGPGGQGPYGPGASAAAAAAGGYGPGSGQQGPGQQGPGQQGPGQQGPGQQGPGQQGPGQQGPGQQGPGQQGPGGQGAYGPGASAAAGAAGGYGPGSGQQGPGQQGPGQQGPGQQGPGQQGPGQQGPGQQGPGQQGPYGPGASAAAAAAGGYGPGSGQQGPGQQGPGQQGPGGQGPYGPGAASAAVSVGGYGPQSSSVPVASAVASRLSSPAASSRVSSAVSSLVSSGPTKHAALSNTISSVVSQVSASNPGLSGCDVLVQALLEVVSALVSILGSSSIGQINYGASAQYTQMVGQSVAQALA

SEQ ID NO: 2 - protein, 410 aa, Araneus diadematus
  PEPTIDE (1)..(410): ADF-4
AGSSAAAAAAASGSGGYGPENQGPSGPVAYGPGGPVSSAAAAAAAGSGPGGYGPENQGPSGPGGYGPGGSGSSAAAAAAAASGPGGYGPGSQGPSGPGGSGGYGPGSQGASGPGGPGASAAAAAAAAAASGPGGYGPGSQGPSGPGAYGPGGPGSSAAAAAAAASGPGGYGPGSQGPSGPGVYGPGGPGSSAAAAAAAGSGPGGYGPENQGPSGPGGYGPGGSGSSAAAAAAAASGPGGYGPGSQGPSGPGGSGGYGPGSQGGSGPGASAAAAAAAASGPGGYGPGSQGPSGPGYQGPSGPGAYGPSPSASASVAASVYLRLQPRLEVSSAVSSLVSSGPTNGAAVSGALNSLVSQISASNPGLSGCDALVQALLELVSALVAILSSASIGQVNVSSVSQSTQMISQALS

SEQ ID NO: 3 - protein, 5 aa, Artificial Sequence
  synthetic
  REPEAT (1)..(5): consensus peptide motif
GPGXX

SEQ ID NO: 4 - protein, 5 aa, Araneus diadematus
  VARIANT (4)..(4): Q at position 4 may also be alanine, serine, glycine, tyrosine, proline, or glutamine
  VARIANT (5)..(5): Q at position 5 may also be alanine, serine, glycine, tyrosine, proline, or glutamine
GPGQQ

SEQ ID NO: 5 - protein, 5 aa, Araneus diadematus
  REPEAT (1)..(5): peptide motif (ADF-3)
GPGAS

SEQ ID NO: 6 - protein, 5 aa, Araneus diadematus
  REPEAT (1)..(5): peptide motif (ADF-3)
GPGSG

SEQ ID NO: 7 - protein, 5 aa, Araneus diadematus
  REPEAT (1)..(5): peptide motif (ADF-4)
GPGGY

SEQ ID NO: 8 - protein, 5 aa, Araneus diadematus
  REPEAT (1)..(5): peptide motif (ADF-4)
GPGGP

SEQ ID NO: 9 - protein, 5 aa, Nephila clavipes
  REPEAT (1)..(5): peptide motif (flagelliform protein)
GPGGA

SEQ ID NO: 10 - protein, 5 aa, Arthropoda
  REPEAT (1)..(5): peptide motif (resilin)
GPGGG

SEQ ID NO: 11 - protein, 5 aa, Nephila clavipes
  REPEAT (1)..(5): peptide motif (flagelliform protein)
GPGGS

SEQ ID NO: 12 - protein, 5 aa, Artificial Sequence
  synthetic
  REPEAT (1)..(5): Ax peptide motif
AAAAA

SEQ ID NO: 13 - protein, 6 aa, Araneus diadematus
  REPEAT (1)..(6): Ax peptide motif (ADF 3)
AAAAAA

SEQ ID NO: 14 - protein, 7 aa, Araneus diadematus
  REPEAT (1)..(7): Ax peptide motif (ADF-4)
AAAAAAA

SEQ ID NO: 15 - protein, 8 aa, Araneus diadematus
  REPEAT (1)..(8): Ax peptide motif (ADF-4)
AAAAAAAA

SEQ ID NO: 16 - protein, 9 aa, Artificial Sequence
  synthetic
  REPEAT (1)..(9): Ax peptide motif
AAAAAAAAA

SEQ ID NO: 17 - protein, 10 aa, Araneus diadematus
  REPEAT (1)..(10): Ax peptide motif (ADF-4)
AAAAAAAAAA

SEQ ID NO: 18 - protein, 9 aa, Arthropoda
  REPEAT (1)..(9): peptide motif (based on resilin)
GGRPSDTYG

SEQ ID NO: 19 - protein, 9 aa, Arthropoda
  REPEAT (1)..(9): peptide motif (based on resilin)
GGRPSSSYG

SEQ ID NO: 20 - protein, 24 aa, Artificial Sequence
  synthetic
  DOMAIN (1)..(24): Module A (ADF-3)
GPYGPGASAAAAAAGGYGPGSGQQ

SEQ ID NO: 21 - protein, 35 aa, Artificial Sequence
  synthetic
  DOMAIN (1)..(35): Module C (ADF-4)
GSSAAAAAAAASGPGGYGPENQGPSGPGGYGPGGP

SEQ ID NO: 22 - protein, 20 aa, Artificial Sequence
  synthetic
  DOMAIN (1)..(20): Module Q (ADF-3)
GPGQQGPGQQGPGQQGPGQQ

SEQ ID NO: 23 - protein, 4 aa, Artificial Sequence
  synthetic
  peptide (1)..(4): peptide linker
GGCG

SEQ ID NO: 24 - protein, 4 aa, Artificial Sequence
  synthetic
  peptide (1)..(4): peptide linker
GCGG

SEQ ID NO: 25 - protein, 34 aa, Artificial Sequence
  synthetic
  DOMAIN (1)..(34): Module S (Resilin)
PGSSAAAAAAAASGPGQGQGQGQGQGGRPSDTYG

SEQ ID NO: 26 - protein, 39 aa, Artificial Sequence
  synthetic
  DOMAIN (1)..(39): Module R (Resilin)
SAAAAAAAAGPGGGNGGRPSDTYGAPGGGNGGRPSSSYG

SEQ ID NO: 27 - protein, 4 aa, Artificial Sequence
  synthetic
  peptide (1)..(4): peptide linker
GGKG

SEQ ID NO: 28 - protein, 4 aa, Artificial Sequence
  synthetic
  peptide (1)..(4): peptide linker
GKGG

SEQ ID NO: 29 - protein, 24 aa, Artificial Sequence
  synthetic
  DOMAIN (1)..(24): Module Ac
GPYGPGASAAAAAAGGYGPGCGQQ

SEQ ID NO: 30 - protein, 24 aa, Artificial Sequence
  synthetic
  DOMAIN (1)..(24): Module Ak
GPYGPGASAAAAAAGGYGPGKGQQ

SEQ ID NO: 31 - protein, 35 aa, Artificial Sequence
  synthetic
  DOMAIN (1)..(35): Module Cc
GSSAAAAAAAASGPGGYGPENQGPCGPGGYGPGGP

SEQ ID NO: 32 - protein, 35 aa, Artificial Sequence
  synthetic
  DOMAIN (1)..(35): Module Ck1
GSSAAAAAAAASGPGGYGPENQGPKGPGGYGPGGP

SEQ ID NO: 33 - protein, 35 aa, Artificial Sequence
  synthetic
  DOMAIN (1)..(35): Module Ck2
GSSAAAAAAAASGPGGYGPKNQGPSGPGGYGPGGP

SEQ ID NO: 34 - protein, 35 aa, Artificial Sequence
  synthetic
  DOMAIN (1)..(35): Module Ckc
GSSAAAAAAAASGPGGYGPKNQGPCGPGGYGPGGP

SEQ ID NO: 35 - protein, 13 aa, Artificial Sequence
  synthetic
  DOMAIN (1)..(13): TAG cys1
GCGGGGGGSGGGG

SEQ ID NO: 36 - protein, 8 aa, Artificial Sequence
  synthetic
  DOMAIN (1)..(8): TAG cys2
GCGGGGGG

SEQ ID NO: 37 - protein, 14 aa, Artificial Sequence
  synthetic
  DOMAIN (1)..(14): TAG cys3
GCGGSGGGGSGGGG

SEQ ID NO: 38 - protein, 13 aa, Artificial Sequence
  synthetic
  DOMAIN (1)..(13): TAG lys1
GKGGGGGGSGGGG

SEQ ID NO: 39 - protein, 8 aa, Artificial Sequence
  synthetic
  DOMAIN (1)..(8): TAG lys2
GKGGGGGG

SEQ ID NO: 40 - protein, 5 aa, Arthropoda
  REPEAT (1)..(5): peptide motif (resilin)
GPGQG

SEQ ID NO: 41 - protein, 124 aa, Artificial Sequence
  based on ADF-3
  DOMAIN (1)..(124): NR3 (ADF-3)
GAASAAVSVGGYGPQSSSAPVASAAASRLSSPAASSRVSSAVSSLVSSGPTNQAALSNTISSVVSQVSASNPGLSGCDVLVQALLEVVSALVSILGSSSIGQINYGASAQYTQMVGQSVAQALA

SEQ ID NO: 42 - protein, 109 aa, Artificial Sequence
  based on ADF-4
  DOMAIN (1)..(109): NR4 (ADF-4)
GAYGPSPSASASVAASRLSSPAASSRVSSAVSSLVSSGPTNGAAVSGALNSLVSQISASNPGLSGCDALVQALLELVSALVAILSSASIGQVNVSSVSQSTQMISQALS

SEQ ID NO: 43 - protein, 747 aa, Araneus diadematus
  PEPTIDE (1)..(747): MaSp I
QGAGAAAAAAGGAGQGGYGGLGGQGAGQGGYGGLGGQGAGQGAGAAAAAAAGGAGQGGYGGLGSQGAGRGGQGAGAAAAAAGGAGQGGYGGLGSQGAGRGGLGGQGAGAAAAAAAGGAGQGGYGGLGNQGAGRGGQGAAAAAAGGAGQGGYGGLGSQGAGRGGLGGQGAGAAAAAAGGAGQGGYGGLGGQGAGQGGYGGLGSQGAGRGGLGGQGAGAAAAAAAGGAGQGGLGGQGAGQGAGASAAAAGGAGQGGYGGLGSQGAGRGGEGAGAAAAAAGGAGQGGYGGLGGQGAGQGGYGGLGSQGAGRGGLGGQGAGAAAAGGAGQGGLGGQGAGQGAGAAAAAAGGAGQGGYGGLGSQGAGRGGLGGQGAGAVAAAAAGGAGQGGYGGLGSQGAGRGGQGAGAAAAAAGGAGQRGYGGLGNQGAGRGGLGGQGAGAAAAAAAGGAGQGGYGGLGNQGAGRGGQGAAAAAGGAGQGGYGGLGSQGAGRGGQGAGAAAAAAVGAGQEGIRGQGAGQGGYGGLGSQGSGRGGLGGQGAGAAAAAAGGAGQGGLGGQGAGQGAGAAAAAAGGVRQGGYGGLGSQGAGRGGQGAGAAAAAAGGAGQGGYGGLGGQGVGRGGLGGQGAGAAAAGGAGQGGYGGVGSGASAASAAASRLSSPQASSRVSSAVSNLVASGPTNSAALSSTISNVVSQIGASNPGLSGCDVLIQALLEVVSALIQILGSSSIGQVNYGSAGQATQIVGQSVYQAL

SEQ ID NO: 44 - protein, 627 aa, Araneus diadematus
  PEPTIDE (1)..(627): MaSp II
PGGYGPGQQGPGGYGPGQQGPSGPGSAAAAAAAAAAGPGGYGPGQQGPGGYGPGQQGPGRYGPGQQGPSGPGSAAAAAAGSGQQGPGGYGPRQQGPGGYGQGQQGPSGPGSAAAASAAASAESGQQGPGGYGPGQQGPGGYGPGQQGPGGYGPGQQGPSGPGSAAAAAAAASGPGQQGPGGYGPGQQGPGGYGPGQQGPSGPGSAAAAAAAASGPGQQGPGGYGPGQQGPGGYGPGQQGLSGPGSAAAAAAAGPGQQGPGGYGPGQQGPSGPGSAAAAAAAAAGPGGYGPGQQGPGGYGPGQQGPSGAGSAAAAAAAGPGQQGLGGYGPGQQGPGGYGPGQQGPGGYGPGSASAAAAAAGPGQQGPGGYGPGQQGPSGPGSASAAAAAAAAGPGGYGPGQQGPGGYAPGQQGPSGPGSASAAAAAAAAGPGGYGPGQQGPGGYAPGQQGPSGPGSAAAAAAAAAGPGGYGPAQQGPSGPGIAASAASAGPGGYGPAQQGPAGYGPGSAVAASAGAGSAGYGPGSQASAAASRLASPDSGARVASAVSNLVSSGPTSSAALSSVISNAVSQIGASNPGLSGCDVLIQALLEIVSACVTILSSSSIGQVNYGAASQFAQVVGQSVLSAF

SEQ ID NO: 45 - protein, 5 aa, artificial sequence
  synthetic
  PEPTIDE (1)..(5): CAMP recognition sequence module
IDAPS

SEQ ID NO: 46 - protein, 12 aa, artificial sequence
  synthetic
  peptide (1)..(12): CAMP recognition sequence module
HHLGGAKQAGDV

SEQ ID NO: 47 - protein, 9 aa, artificial sequence
  synthetic
  peptide (1)..(9): CAMP recognition sequence module
CDPGYIGSR

SEQ ID NO: 48 - protein, 8 aa, artificial sequence
  synthetic
  peptide (1)..(8): CAMP recognition sequence module
AEIDGIEL

SEQ ID NO: 49 - protein, 4 aa, artificial sequence
  synthetic
  peptide (1)..(4): CAMP recognition sequence module
QIDS

SEQ ID NO: 50 - protein, 4 aa, artificial sequence
  synthetic
  peptide (1)..(4): CAMP recognition sequence module
RGDS

SEQ ID NO: 51 - protein, 5 aa, artificial sequence
  synthetic
  peptide (1)..(5): CAMP recognition sequence module
GRGDS

SEQ ID NO: 52 - protein, 5 aa, artificial sequence
  synthetic
  peptide (1)..(5): CAMP recognition sequence module
GRGDY

SEQ ID NO: 53 - protein, 11 aa, artificial sequence
  synthetic
  peptide (1)..(11): CAMP recognition sequence module
GGSGGRGDSPG

SEQ ID NO: 54 - protein, 10 aa, artificial sequence
  synthetic
  peptide (1)..(10): CAMP recognition sequence module
RGDSPASSKP

SEQ ID NO: 55 - protein, 14 aa, artificial sequence
  synthetic
  peptide (1)..(14): CAMP recognition sequence module
CGGNGEPRGDYRAY

SEQ ID NO: 56 - protein, 6 aa, artificial sequence
  synthetic
  peptide (1)..(6): CAMP recognition sequence module Pro = Hydroxyproline (O)
GFPGER

SEQ ID NO: 57 - protein, 6 aa, artificial sequence
  synthetic
  peptide (1)..(6): CAMP recognition sequence module Pro = Hydroxyproline (O)
GLPGER

SEQ ID NO: 58 - protein, 6 aa, artificial sequence
  synthetic
  peptide (1)..(6): CAMP recognition sequence module
GASGER

SEQ ID NO: 59 - protein, 6 aa, artificial sequence
  synthetic
  peptide (1)..(6): CAMP recognition sequence module Pro = Hydroxyproline (O)
GRPGER

SEQ ID NO: 60 - protein, 6 aa, artificial sequence
  synthetic
  peptide (1)..(6): CAMP recognition sequence module Pro = Hydroxyproline (O)
GMPGER

SEQ ID NO: 61 - protein, 6 aa, artificial sequence
  synthetic
  peptide (1)..(6): CAMP recognition sequence module
GLSGER

SEQ ID NO: 62 - protein, 6 aa, artificial sequence
  synthetic
  peptide (1)..(6): CAMP recognition sequence module Pro = Hydroxyproline (O)
GAPGER

SEQ ID NO: 63 - protein, 6 aa, artificial sequence
  synthetic
  peptide (1)..(6): CAMP recognition sequence module Pro = Hydroxyproline (O)
GFPGEK

SEQ ID NO: 64 - protein, 6 aa, artificial sequence
  synthetic
  peptide (1)..(6): CAMP recognition sequence module Pro = Hydroxyproline (O)
GLPGEK

SEQ ID NO: 65 - protein, 6 aa, artificial sequence
  synthetic
  peptide (1)..(6): CAMP recognition sequence module
GASGEK

SEQ ID NO: 66 - protein, 6 aa, artificial sequence
  synthetic
  peptide (1)..(6): CAMP recognition sequence module Pro = Hydroxyproline (O)
GRPGEK

SEQ ID NO: 67 - protein, 6 aa, artificial sequence
  synthetic
  peptide (1)..(6): CAMP recognition sequence module Pro = Hydroxyproline (O)
GMPGEK

SEQ ID NO: 68 - protein, 6 aa, artificial sequence
  synthetic
  peptide (1)..(6): CAMP recognition sequence module
GLSGEK

SEQ ID NO: 69 - protein, 6 aa, artificial sequence
  synthetic
  peptide (1)..(6): CAMP recognition sequence module Pro = Hydroxyproline (O)
GAPGEK

SEQ ID NO: 70 - protein, 6 aa, artificial sequence
  synthetic
  peptide (1)..(6): CAMP recognition sequence module Pro = Hydroxyproline (O)
GLPGEN

SEQ ID NO: 71 - protein, 6 aa, artificial sequence
  synthetic
  peptide (1)..(6): CAMP recognition sequence module
GLKGEN

SEQ ID NO: 72 - DNA, 39 bp, artificial sequence
  synthetic oligonucleotide for the RGD-tag
  oligonucleotide (1)..(39)
gatccatgggcggtcgtggtgactctccgggttaatgaa

SEQ ID NO: 73 - DNA, 39 bp, artificial sequence
  synthetic oligonucleotide for the RGD-tag
  oligonucleotide (1)..(39)
agctttcattaacccggagagtcaccacgaccgcccatg

SEQ ID NO: 74 - DNA, 30 bp, artificial sequence
  synthetic oligonucleotide for the spacer sequence
  oligonucleotide (1)..(30)
gatccatgggcggtggctctggttaatgaa

SEQ ID NO: 75 - DNA, 30 bp, artificial sequence
  synthetic oligonucleotide for the spacer sequence
  oligonucleotide (1)..(30)
agctttcattaaccagagccaccgcccatg

SEQ ID NO: 76 - protein, 136 aa, artificial
  synthetic
  domain (1)..(136): derived from Latrodectus hesperus
MGQANTPWSSKANADAFINSFISAASNTGSFSQDQMEDMSLIGNTLMAAMDNMGGRITPSKLQALDMAFASSVAEIAASEGGDLGVTTNAIADALTSAFYQTTGVVNSRFISEIRSLIGMFAQASANDVYASAGSG

SEQ ID NO: 77 - protein, 137 aa, artificial
  synthetic
  domain (1)..(137): derived from Latrodectus hesperus
MGQANTPWSSKENADAFIGAFMNAASQSGAFSSDQIDDMSVISNTLMAAMDNMGGRITQSKLQALDMAFASSVAEIAVADGQNVGAATNAISDALRSAFYQTTGVVNNQFITGISSLIGMFAQVSGNEVSYSSAGSG

SEQ ID NO: 78 - protein, 587 aa, artificial
  synthetic
  Protein (1)..(587): C16spRGD with T7 TAG
MASMTGGQQMGRGSMGSSAAAAAAAASGPGGYGPENQGPSGPGGYGPGGPGSSAAAAAAAASGPGGYGPENQGPSGPGGYGPGGPGSSAAAAAAAASGPGGYGPENQGPSGPGGYGPGGPGSSAAAAAAAASGPGGYGPENQGPSGPGGYGPGGPGSSAAAAAAAASGPGGYGPENQGPSGPGGYGPGGPGSSAAAAAAAASGPGGYGPENQGPSGPGGYGPGGPGSSAAAAAAAASGPGGYGPENQGPSGPGGYGPGGPGSSAAAAAAAASGPGGYGPENQGPSGPGGYGPGGPGSSAAAAAAAASGPGGYGPENQGPSGPGGYGPGGPGSSAAAAAAAASGPGGYGPENQGPSGPGGYGPGGPGSSAAAAAAAASGPGGYGPENQGPSGPGGYGPGGPGSSAAAAAAAASGPGGYGPENQGPSGPGGYGPGGPGSSAAAAAAAASGPGGYGPENQGPSGPGGYGPGGPGSSAAAAAAAASGPGGYGPENQGPSGPGGYGPGGPGSSAAAAAAAASGPGGYGPENQGPSGPGGYGPGGPGSSAAAAAAAASGPGGYGPENQGPSGPGGYGPGGPGGGSGGRGDSPG